European Patent Specification EP 4 108 248 B1, published September 17, 2025. Title: C. NOVYI FOR THE TREATMENT OF SOLID TUMORS IN HUMANS. Applicant: BIOMED VALLEY DISCOVERIES, INC. THE JOHNS HOPKINS UNIVERSITY. The sequence listing filed with the application follows.

SEQUENCE LISTING (170 sequences)

SEQ ID NO: 1 - DNA, 11 bp, Canis familiaris
  misc_feature (6)..(6): C or T
ccctanctggg

SEQ ID NO: 2 - DNA, 11 bp, Canis familiaris
  misc_feature (6)..(6): G or T
aaaacntccag

SEQ ID NO: 3 - DNA, 11 bp, Canis familiaris
  misc_feature (6)..(6): T or A
ggtcantatta

SEQ ID NO: 4 - DNA, 11 bp, Canis familiaris
  misc_feature (6)..(6): C or T
aggagngacgc

SEQ ID NO: 5 - DNA, 11 bp, Canis familiaris
  misc_feature (6)..(6): G or T
gcccgngatgg

SEQ ID NO: 6 - DNA, 11 bp, Canis familiaris
  misc_feature (6)..(6): C or T
cgcacncacct

SEQ ID NO: 7 - DNA, 11 bp, Canis familiaris
  misc_feature (6)..(6): T or G
ttaccncaatc

SEQ ID NO: 8 - DNA, 11 bp, Canis familiaris
  misc_feature (6)..(6): T or G
aacaangtcat

SEQ ID NO: 9 - DNA, 11 bp, Canis familiaris
  misc_feature (6)..(6): G or A
ccgtgntgagt

SEQ ID NO: 10 - DNA, 11 bp, Canis familiaris
  misc_feature (6)..(6): C or T
acaagncggcc

SEQ ID NO: 11 - DNA, 11 bp, Canis familiaris
  misc_feature (6)..(6): C or T
atctgcggttc

SEQ ID NO: 12 - DNA, 11 bp, Canis familiaris
  misc_feature (6)..(6): G or A
gattcggaagt

SEQ ID NO: 13 - DNA, 11 bp, Canis familiaris
  misc_feature (6)..(6): C or G
acctactttga

SEQ ID NO: 14 - DNA, 11 bp, Canis familiaris
  misc_feature (6)..(6): C or T
tgtcacactca

SEQ ID NO: 15 - DNA, 11 bp, Canis familiaris
  misc_feature (6)..(6): A or G
aagcanagcac

SEQ ID NO: 16 - DNA, 11 bp, Canis familiaris
  misc_feature (6)..(6): A or C
agttgntggac

SEQ ID NO: 17 - DNA, 11 bp, Canis familiaris
  misc_feature (6)..(6): A or G
cctgangaatt

SEQ ID NO: 18 - DNA, 11 bp, Canis familiaris
  misc_feature (6)..(6): G or A
tcttgnagaag

SEQ ID NO: 19 - DNA, 11 bp, Canis familiaris
  misc_feature (6)..(6): A or C
acccanagatg

SEQ ID NO: 20 - DNA, 11 bp, Canis familiaris
  misc_feature (6)..(6): A or G
ctgggncttac

SEQ ID NO: 21 - DNA, 11 bp, Canis familiaris
  misc_feature (6)..(6): C or absent
aggtanagcag

SEQ ID NO: 22 - DNA, 11 bp, Canis familiaris
  misc_feature (6)..(6): A or T
atcgangtcaa

SEQ ID NO: 23 - DNA, 13 bp, Canis familiaris
  misc_feature (6)..(8): TGC or absent
gctgtnnngctgc

SEQ ID NO: 24 - DNA, 11 bp, Canis familiaris
  misc_feature (6)..(6): G or A
agacangcccc

SEQ ID NO: 25 - DNA, 11 bp, Canis familiaris
  misc_feature (6)..(6): T or absent
cggtcncccag

SEQ ID NO: 26 - DNA, 11 bp, Canis familiaris
  misc_feature (6)..(6): C or T
gaaggncttct

SEQ ID NO: 27 - DNA, 11 bp, Canis familiaris
  misc_feature (6)..(6): C or T
aggcgngcaca

SEQ ID NO: 28 - DNA, 11 bp, Canis familiaris
  misc_feature (6)..(6): T or absent
gaagantttgg

SEQ ID NO: 29 - DNA, 11 bp, Canis familiaris
  misc_feature (6)..(6): A or T
tttggntttat

SEQ ID NO: 30 - DNA, 11 bp, Canis familiaris
  misc_feature (6)..(6): C or T
ttcggnggcgg

SEQ ID NO: 31 - DNA, 11 bp, Canis familiaris
  misc_feature (6)..(6): C or T
cccccncagtg

SEQ ID NO: 32 - DNA, 11 bp, Canis familiaris
  misc_feature (6)..(6): C or T
tttttnctcgg

SEQ ID NO: 33 - DNA, 11 bp, Canis familiaris
  misc_feature (6)..(6): C or T
ccaccngctca

SEQ ID NO: 34 - DNA, 11 bp, Canis familiaris
  misc_feature (6)..(6): G or T
attacngcagc

SEQ ID NO: 35 - DNA, 11 bp, Canis familiaris
  misc_feature (6)..(6): C or G
atcacnccgga

SEQ ID NO: 36 - DNA, 11 bp, Canis familiaris
  misc_feature (6)..(6): C or T
gacatnctcta

SEQ ID NO: 37 - DNA, 11 bp, Canis familiaris
  misc_feature (6)..(6): C or T
aatgcnaccag

SEQ ID NO: 38 - DNA, 11 bp, Canis familiaris
  misc_feature (6)..(6): C or T
cagctngccca

SEQ ID NO: 39 - DNA, 11 bp, Canis familiaris
  misc_feature (6)..(6): G or A
gggggncaggc

SEQ ID NO: 40 - DNA, 11 bp, Canis familiaris
  misc_feature (6)..(6): C or T
cacttnaggaa

SEQ ID NO: 41 - DNA, 11 bp, Canis familiaris
  misc_feature (6)..(6): C or T
gggctncttcc

SEQ ID NO: 42 - DNA, 11 bp, Canis familiaris
  misc_feature (6)..(6): G or A
tgatantacta

SEQ ID NO: 43 - DNA, 11 bp, Canis familiaris
  misc_feature (6)..(6): G or A
ctcctngtctc

SEQ ID NO: 44 - DNA, 11 bp, Canis familiaris
  misc_feature (6)..(6): C or T
ttcaancatgt

SEQ ID NO: 45 - DNA, 11 bp, Canis familiaris
  misc_feature (6)..(6): C or T
catttntttgc

SEQ ID NO: 46 - DNA, 11 bp, Canis familiaris
  misc_feature (6)..(6): C or T
aatgtncgtgc

SEQ ID NO: 47 - DNA, 11 bp, Canis familiaris
  misc_feature (6)..(6): C or T
ggcccnccatg

SEQ ID NO: 48 - DNA, 11 bp, Canis familiaris
  misc_feature (6)..(6): C or T
attttngggac

SEQ ID NO: 49 - DNA, 11 bp, Canis familiaris
  misc_feature (6)..(6): C or T
agatgncccat

SEQ ID NO: 50 - DNA, 11 bp, Canis familiaris
  misc_feature (6)..(6): C or T
aactcnctgcg

SEQ ID NO: 51 - DNA, 11 bp, Canis familiaris
  misc_feature (6)..(6): C or T
attttnttgaa

SEQ ID NO: 52 - DNA, 11 bp, Canis familiaris
  misc_feature (6)..(6): G or T
aaccanccttc

SEQ ID NO: 53 - DNA, 11 bp, Canis familiaris
  misc_feature (6)..(6): G or A
tcagangcaga

SEQ ID NO: 54 - DNA, 11 bp, Canis familiaris
  misc_feature (6)..(6): C or T
agaaanccctc

SEQ ID NO: 55 - DNA, 11 bp, Canis familiaris
  misc_feature (6)..(6): C or T
tgcatngacat

SEQ ID NO: 56 - DNA, 11 bp, Canis familiaris
  misc_feature (6)..(6): G or A
agtggngccgg

SEQ ID NO: 57 - DNA, 11 bp, Canis familiaris
  misc_feature (6)..(6): C or T
tcattnttcgg

SEQ ID NO: 58 - DNA, 11 bp, Canis familiaris
  misc_feature (6)..(6): G or A
tctggnaatgg

SEQ ID NO: 59 - DNA, 11 bp, Canis familiaris
  misc_feature (6)..(6): C or T
gacttngccca

SEQ ID NO: 60 - DNA, 11 bp, Canis familiaris
  misc_feature (6)..(6): C or T
gttttncttct

SEQ ID NO: 61 - DNA, 11 bp, Canis familiaris
  misc_feature (6)..(6): C or T
attgtncaaga

SEQ ID NO: 62 - DNA, 11 bp, Canis familiaris
  misc_feature (6)..(6): C or T
ggctgntgaag

SEQ ID NO: 63 - DNA, 11 bp, Canis familiaris
  misc_feature (6)..(6): G or A
ggtganagtcc

SEQ ID NO: 64 - DNA, 11 bp, Canis familiaris
  misc_feature (6)..(6): C or A
ggctgnccaga

SEQ ID NO: 65 - DNA, 11 bp, Canis familiaris
  misc_feature (6)..(6): C or T
cggggncccgg

SEQ ID NO: 66 - DNA, 11 bp, Canis familiaris
  misc_feature (6)..(6): G or A
ccaagnaaatt

SEQ ID NO: 67 - DNA, 11 bp, Canis familiaris
  misc_feature (6)..(6): C or T
aaattncctac

SEQ ID NO: 68 - DNA, 11 bp, Canis familiaris
  misc_feature (6)..(6): G or A
tgcacnaagct

SEQ ID NO: 69 - DNA, 11 bp, Canis familiaris
  misc_feature (6)..(6): G or A
tttggnaatca

SEQ ID NO: 70 - DNA, 11 bp, Canis familiaris
  misc_feature (6)..(6): C or T
tctcancatag

SEQ ID NO: 71 - DNA, 11 bp, Canis familiaris
  misc_feature (6)..(6): C or T
aatttncatag

SEQ ID NO: 72 - DNA, 11 bp, Canis familiaris
  misc_feature (6)..(6): C or T
aagganggagg

SEQ ID NO: 73 - DNA, 11 bp, Canis familiaris
  misc_feature (6)..(6): C or T
attttnatttt

SEQ ID NO: 74 - DNA, 11 bp, Canis familiaris
  misc_feature (6)..(6): C or T
cctccnctgtg

SEQ ID NO: 75 - DNA, 11 bp, Canis familiaris
  misc_feature (6)..(6): C or T
gctgtntggag

SEQ ID NO: 76 - DNA, 11 bp, Canis familiaris
  misc_feature (6)..(6): G or A
agactnatctc

SEQ ID NO: 77 - DNA, 11 bp, Canis familiaris
  misc_feature (6)..(6): G or A
gggaanagaag

SEQ ID NO: 78 - DNA, 11 bp, Canis familiaris
  misc_feature (6)..(6): C or T
cttccngcttg

SEQ ID NO: 79 - DNA, 11 bp, Canis familiaris
  misc_feature (6)..(6): G or A
aatacnaacaa

SEQ ID NO: 80 - DNA, 11 bp, Canis familiaris
  misc_feature (6)..(6): G or A
tgttgnatgtt

SEQ ID NO: 81 - DNA, 11 bp, Canis familiaris
  misc_feature (6)..(6): G or A
tgtcgnagcgc

SEQ ID NO: 82 - DNA, 11 bp, Canis familiaris
  misc_feature (6)..(6): C or T
gtgccngtcca

SEQ ID NO: 83 - DNA, 11 bp, Canis familiaris
  misc_feature (6)..(6): G or A
gatccngtctc

SEQ ID NO: 84 - DNA, 11 bp, Canis familiaris
  misc_feature (6)..(6): C or T
cgactncccca

SEQ ID NO: 85 - DNA, 11 bp, Canis familiaris
  misc_feature (6)..(6): C or T
tggtcnagcta

SEQ ID NO: 86 - DNA, 11 bp, Canis familiaris
  misc_feature (6)..(6): C or T
ccgagntcatg

SEQ ID NO: 87 - DNA, 11 bp, Canis familiaris
  misc_feature (6)..(6): G or A
ctgtcnaatgt

SEQ ID NO: 88 - DNA, 11 bp, Canis familiaris
  misc_feature (6)..(6): G or A
ccacgnagtca

SEQ ID NO: 89 - DNA, 11 bp, Canis familiaris
  misc_feature (6)..(6): G or A
gttctnaacta

SEQ ID NO: 90 - DNA, 11 bp, Canis familiaris
  misc_feature (6)..(6): G or A
gggagnagaaa

SEQ ID NO: 91 - DNA, 11 bp, Canis familiaris
  misc_feature (6)..(6): C or T
aaaatnatgca

SEQ ID NO: 92 - DNA, 11 bp, Canis familiaris
  misc_feature (6)..(6): G or A
taaacnatcag

SEQ ID NO: 93 - DNA, 11 bp, Canis familiaris
  misc_feature (6)..(6): G or A
ggcatnatggc

SEQ ID NO: 94 - DNA, 11 bp, Canis familiaris
  misc_feature (6)..(6): C or T
caattngccag

SEQ ID NO: 95 - DNA, 11 bp, Canis familiaris
  misc_feature (6)..(6): G or A
ttttgnaaatt

SEQ ID NO: 96 - DNA, 11 bp, Canis familiaris
  misc_feature (6)..(6): C or A
cacttnggagc

SEQ ID NO: 97 - DNA, 11 bp, Canis familiaris
  misc_feature (6)..(6): G or A
cttctngaggg

SEQ ID NO: 98 - DNA, 11 bp, Canis familiaris
  misc_feature (6)..(6): C or T
gatttnctctg

SEQ ID NO: 99 - DNA, 11 bp, Canis familiaris
  misc_feature (6)..(6): C or T
ctactngtgag

SEQ ID NO: 100 - DNA, 11 bp, Canis familiaris
  misc_feature (6)..(6): G or C
gttcanctcaa

SEQ ID NO: 101 - DNA, 11 bp, Canis familiaris
  misc_feature (6)..(6): G or A
gacatnaaatt

SEQ ID NO: 102 - DNA, 11 bp, Canis familiaris
  misc_feature (6)..(6): C or T
gatttncaagt

SEQ ID NO: 103 - DNA, 11 bp, Canis familiaris
  misc_feature (6)..(6): G or A
tggganatgtc

SEQ ID NO: 104 - DNA, 11 bp, Canis familiaris
  misc_feature (6)..(6): C or T
acttantttat

SEQ ID NO: 105 - DNA, 11 bp, Canis familiaris
  misc_feature (6)..(6): G or A
tcactnagttg

SEQ ID NO: 106 - DNA, 11 bp, Canis familiaris
  misc_feature (6)..(6): G or A
ggacgncagcg

SEQ ID NO: 107 - DNA, 11 bp, Canis familiaris
  misc_feature (6)..(6): C or T
tttttncgtct

SEQ ID NO: 108 - DNA, 11 bp, Canis familiaris
  misc_feature (6)..(6): T or C
taaacntgcac

SEQ ID NO: 109 - DNA, 11 bp, Canis familiaris
  misc_feature (6)..(6): C or T
aactcntcaac

SEQ ID NO: 110 - DNA, 11 bp, Canis familiaris
  misc_feature (6)..(6): G or A
ccagcnacagc

SEQ ID NO: 111 - DNA, 11 bp, Canis familiaris
  misc_feature (6)..(6): A or T
gaaatnttata

SEQ ID NO: 112 - DNA, 11 bp, Canis familiaris
  misc_feature (6)..(6): C or T
ggtccnccggc

SEQ ID NO: 113 - DNA, 11 bp, Canis familiaris
  misc_feature (6)..(6): G or A
aatcanaaaga

SEQ ID NO: 114 - DNA, 11 bp, Canis familiaris
  misc_feature (6)..(6): G or A
gccatnatctg

SEQ ID NO: 115 - DNA, 11 bp, Canis familiaris
  misc_feature (6)..(6): G or A
tcttcnaagca

SEQ ID NO: 116 - DNA, 11 bp, Canis familiaris
  misc_feature (6)..(6): C or T
gtcttngggtg

SEQ ID NO: 117 - DNA, 11 bp, Canis familiaris
  misc_feature (6)..(6): C or T
agtttncatag

SEQ ID NO: 118 - DNA, 11 bp, Canis familiaris
  misc_feature (6)..(6): G or A
ttgatnaacat

SEQ ID NO: 119 - DNA, 11 bp, Canis familiaris
  misc_feature (6)..(6): C or T
cttttnataat

SEQ ID NO: 120 - DNA, 11 bp, Canis familiaris
  misc_feature (6)..(6): C or T
tgactntcttg

SEQ ID NO: 121 - DNA, 11 bp, Canis familiaris
  misc_feature (6)..(6): G or A
ggatgntctta

SEQ ID NO: 122 - DNA, 11 bp, Canis familiaris
  misc_feature (6)..(6): G or A
agggcnaagtt

SEQ ID NO: 123 - DNA, 11 bp, Canis familiaris
  misc_feature (6)..(6): A or C
gcatcncctca

SEQ ID NO: 124 - DNA, 11 bp, Canis familiaris
  misc_feature (6)..(6): G or C
cgtttnttaca

SEQ ID NO: 125 - DNA, 11 bp, Canis familiaris
  misc_feature (6)..(6): G or A
tggganaggcg

SEQ ID NO: 126 - DNA, 11 bp, Canis familiaris
  misc_feature (6)..(6): C or T
actttntttaa

SEQ ID NO: 127 - DNA, 11 bp, Canis familiaris
  misc_feature (6)..(6): G or A
gaccgnttcgc

SEQ ID NO: 128 - DNA, 11 bp, Canis familiaris
  misc_feature (6)..(6): C or T
gttttntgcat

SEQ ID NO: 129 - DNA, 11 bp, Canis familiaris
  misc_feature (6)..(6): C or T
gttctngtgac

SEQ ID NO: 130 - DNA, 11 bp, Canis familiaris
  misc_feature (6)..(6): G or A
gggagnaaaaa

SEQ ID NO: 131 - DNA, 11 bp, Canis familiaris
  misc_feature (6)..(6): C or T
tgtggncttgt

SEQ ID NO: 132 - DNA, 11 bp, Canis familiaris
  misc_feature (6)..(6): G or A
cggccngaggc

SEQ ID NO: 133 - DNA, 11 bp, Canis familiaris
  misc_feature (6)..(6): G or A
tggacncgggc

SEQ ID NO: 134 - DNA, 11 bp, Canis familiaris
  misc_feature (6)..(6): G or A
tcttcntctcc

SEQ ID NO: 135 - DNA, 11 bp, Canis familiaris
  misc_feature (6)..(6): T or absent
gggtgnttttt

SEQ ID NO: 136 - DNA, 11 bp, Canis familiaris
  misc_feature (6)..(6): A or G
aaaggnctgga

SEQ ID NO: 137 - DNA, 14 bp, Canis familiaris
  misc_feature (6)..(9): GATG or absent
aagatnnnnatgta

SEQ ID NO: 138 - DNA, 11 bp, Canis familiaris
  misc_feature (6)..(6): A or G
cctcanagctg

SEQ ID NO: 139 - DNA, 11 bp, Canis familiaris
  misc_feature (6)..(6): C or T
ctcggnggctc

SEQ ID NO: 140 - DNA, 11 bp, Canis familiaris
  misc_feature (6)..(6): C or T
cattcnctctt

SEQ ID NO: 141 - DNA, 11 bp, Canis familiaris
  misc_feature (6)..(6): T or C
tctttntgctg

SEQ ID NO: 142 - DNA, 11 bp, Canis familiaris
  misc_feature (6)..(6): G or A
aactgntataa

SEQ ID NO: 143 - DNA, 11 bp, Canis familiaris
  misc_feature (6)..(6): G or T
tttcanttttg

SEQ ID NO: 144 - DNA, 11 bp, Canis familiaris
  misc_feature (6)..(6): C or A
tccagnccagt

SEQ ID NO: 145 - DNA, 11 bp, Canis familiaris
  misc_feature (6)..(6): G or A
gagagncgggg

SEQ ID NO: 146 - DNA, 11 bp, Canis familiaris
  misc_feature (6)..(6): C or T
gtgcangtggg

SEQ ID NO: 147 - DNA, 11 bp, Canis familiaris
  misc_feature (6)..(6): G or C
agggcnccccg

SEQ ID NO: 148 - DNA, 11 bp, Canis familiaris
  misc_feature (6)..(6): G or A
ccttcnccttt

SEQ ID NO: 149 - DNA, 11 bp, Canis familiaris
  misc_feature (6)..(6): G or A
caggangcccc

SEQ ID NO: 150 - DNA, 11 bp, Canis familiaris
  misc_feature (6)..(6): C or T
cagggngaatg

SEQ ID NO: 151 - DNA, 11 bp, Canis familiaris
  misc_feature (6)..(6): C or A
tggccncctgc

SEQ ID NO: 152 - DNA, 11 bp, Canis familiaris
  misc_feature (6)..(6): G or A
ctgatnctgcc

SEQ ID NO: 153 - DNA, 11 bp, Canis familiaris
  misc_feature (6)..(6): C or T
cagcanaggcc

SEQ ID NO: 154 - DNA, 11 bp, Canis familiaris
  misc_feature (6)..(6): G or A
tgggcntggcc

SEQ ID NO: 155 - DNA, 11 bp, Canis familiaris
  misc_feature (6)..(6): C or T
tcaggnggcac

SEQ ID NO: 156 - DNA, 11 bp, Canis familiaris
  misc_feature (6)..(6): G or A
ccacanctccc

SEQ ID NO: 157 - DNA, 11 bp, Canis familiaris
  misc_feature (6)..(6): C or T
ccgagntgccg

SEQ ID NO: 158 - DNA, 11 bp, Canis familiaris
  misc_feature (6)..(6): G or A
ctgtancttcg

SEQ ID NO: 159 - DNA, 11 bp, Canis familiaris
  misc_feature (6)..(6): G or A
gctccnatgag

SEQ ID NO: 160 - DNA, 11 bp, Canis familiaris
  misc_feature (6)..(6): G or A
actcgntgatg

SEQ ID NO: 161 - DNA, 11 bp, Canis familiaris
  misc_feature (6)..(6): G or absent
aaagtnggggg

SEQ ID NO: 162 - DNA, 11 bp, Canis familiaris
  misc_feature (6)..(6): C or A
ggaaanaagac

SEQ ID NO: 163 - DNA, 11 bp, Canis familiaris
  misc_feature (6)..(6): A or G
acaggncgtag

SEQ ID NO: 164 - DNA, 11 bp, Canis familiaris
  misc_feature (6)..(6): C or T
ggcagntgcgg

SEQ ID NO: 165 - DNA, 11 bp, Canis familiaris
  misc_feature (6)..(6): G or A
ccccgnctcct

SEQ ID NO: 166 - DNA, 11 bp, Canis familiaris
  misc_feature (6)..(6): C or T
actgcnacaac

SEQ ID NO: 167 - DNA, 11 bp, Canis familiaris
  misc_feature (6)..(6): C or T
ccctgnaggag

SEQ ID NO: 168 - DNA, 11 bp, Canis familiaris
  misc_feature (6)..(6): G or A
ggaaanctact

SEQ ID NO: 169 - DNA, 11 bp, Canis familiaris
  misc_feature (6)..(6): C or T
catgantgtcc

SEQ ID NO: 170 - DNA, 11 bp, Canis familiaris
  misc_feature (6)..(6): C or T
cttcgntcaag